European Patent Application EP 4 772 523 A1, published July 8, 2026. Title: D-form of peptides and use thereof. Applicant: Hirosaki University. The sequence listing filed with the application follows.

SEQUENCE LISTING (40 sequences)

SEQ ID NO: 1 - protein, 7 aa, synthetic construct
  REGION 1..7: note = D-amino acids
  SITE 1: note = X can be His or Gln
  SITE 2: note = X can be Pro or Ser
  SITE 3: note = X can be Asn or Lys
XXXEVRS

SEQ ID NO: 2 - protein, 7 aa, synthetic construct
  REGION 1..7: note = D-amino acids
  SITE 2: note = X can be Try or Leu
  SITE 5: note = X can be Asn, Lys or Try
QXATXLK

SEQ ID NO: 3 - protein, 7 aa, synthetic construct
  REGION 1..7: note = D-amino acids
  SITE 1: note = X can be Ser or Arg
  SITE 4: note = X can be Arg or Trp
  SITE 5: note = X can be Asn or Ile
XTSXXTL

SEQ ID NO: 4 - protein, 7 aa, synthetic construct
  REGION 1..7: note = D-amino acids
XXNEVRS

SEQ ID NO: 5 - protein, 7 aa, synthetic construct
  REGION 1..7: note = D-amino acids
HPNEVRS

SEQ ID NO: 6 - protein, 7 aa, synthetic construct
  REGION 1..7: note = D-amino acids
QPNEVRS

SEQ ID NO: 7 - protein, 7 aa, synthetic construct
  REGION 1..7: note = D-amino acids
HSNEVRS

SEQ ID NO: 8 - protein, 7 aa, synthetic construct
  REGION 1..7: note = D-amino acids
QSNEVRS

SEQ ID NO: 9 - protein, 7 aa, synthetic construct
  REGION 1..7: note = D-amino acids
QPKEVRS

SEQ ID NO: 10 - protein, 7 aa, synthetic construct
  REGION 1..7: note = D-amino acids
HPNEVRS

SEQ ID NO: 11 - protein, 7 aa, synthetic construct
  REGION 1..7: note = D-amino acids
QYATNLK

SEQ ID NO: 12 - protein, 7 aa, synthetic construct
  REGION 1..7: note = D-amino acids
QYATKLK

SEQ ID NO: 13 - protein, 7 aa, synthetic construct
  REGION 1..7: note = D-amino acids
QLATYLK

SEQ ID NO: 14 - protein, 7 aa, synthetic construct
  REGION 1..7: note = D-amino acids
QYATNLK

SEQ ID NO: 15 - protein, 7 aa, synthetic construct
  REGION 1..7: note = D-amino acids
STSRNTL

SEQ ID NO: 16 - protein, 7 aa, synthetic construct
  REGION 1..7: note = D-amino acids
RTSWITL

SEQ ID NO: 17 - protein, 7 aa, synthetic construct
  REGION 1..7: note = D-amino acids
STSRNTL

SEQ ID NO: 18 - protein, 7 aa, synthetic construct
  REGION 1..7: note = D-amino acids
SRVENPH

SEQ ID NO: 19 - protein, 7 aa, synthetic construct
SRVENPQ

SEQ ID NO: 20 - protein, 7 aa, synthetic construct
SRVENSH

SEQ ID NO: 21 - protein, 7 aa, synthetic construct
SRVENSQ

SEQ ID NO: 22 - protein, 7 aa, synthetic construct
SRVEKPQ

SEQ ID NO: 23 - protein, 7 aa, synthetic construct
KLNTAYQ

SEQ ID NO: 24 - protein, 7 aa, synthetic construct
KLKTAYQ

SEQ ID NO: 25 - protein, 7 aa, synthetic construct
KLYTALQ

SEQ ID NO: 26 - protein, 7 aa, synthetic construct
LTNRSTS

SEQ ID NO: 27 - protein, 7 aa, synthetic construct
LTIWSTR

SEQ ID NO: 28 - protein, 15 aa, synthetic construct
MAMVSEFLKQAWFIE

SEQ ID NO: 29 - protein, 15 aa, synthetic construct
  REGION 1..15: note = D-amino acids
MAMVSEFLKQAWFIE

SEQ ID NO: 30 - protein, 7 aa, synthetic construct
HPNEVRS

SEQ ID NO: 31 - protein, 7 aa, synthetic construct
  REGION 1..7: note = D-amino acids
HPNEVRS

SEQ ID NO: 32 - protein, 7 aa, synthetic construct
STSRNTL

SEQ ID NO: 33 - protein, 7 aa, synthetic construct
QYATNLK

SEQ ID NO: 34 - protein, 7 aa, synthetic construct
  REGION 1..7: note = D-amino acids
STSRNTL

SEQ ID NO: 35 - protein, 7 aa, synthetic construct
  REGION 1..7: note = D-amino acids
QYATNLK

SEQ ID NO: 36 - protein, 7 aa, synthetic construct
QPNEVRS

SEQ ID NO: 37 - protein, 7 aa, synthetic construct
HSNEVRS

SEQ ID NO: 38 - protein, 7 aa, synthetic construct
QSNEVRS

SEQ ID NO: 39 - protein, 7 aa, synthetic construct
RRQRRAP

SEQ ID NO: 40 - protein, 8 aa, synthetic construct
IFLLWQRK